European Patent Application EP 4 755 869 A1, published June 10, 2026. Title: ORGANIC COMPOUND. Applicant: Givaudan SA. The sequence listing filed with the application follows.

SEQUENCE LISTING (10 sequences)

SEQ ID NO: 1 - DNA, 945 bp, synthetic construct
  source 1..945: mol_type = other DNA; note = OR2J2 DNA sequence with an optimized C-terminus
atgatgattaaaaaaaatgcaagttcggaagacttctttattctacttggattttctaattggcctcagctggaagtagttctctttgtggttatcttgatcttctacctgatgacactgacaggaaacctgttcatcatcatcctgtcatacgtggactcccatctccacacaccaatgtacttcttcctttcaaacctctcatttctggatctctgctacaccaccagctctatccctcagttgctggtgaatctccggggcccggaaaagaccatctcgtatgctggttgcatggttcaactttactttgttcttgcactgggaatcgcagagtgtgtcctactggtggtgatgtcgtatgatcgttatgtagctgtgtgtagacctttgcattacactgtcctcatgcaccctcgtttctgccacttgttggttgcggcttcttgggtaattggttttactatctcagcacttcattcctcctttactttctgggtacccctttgtggacatcgcctagtggatcacttcttctgtgaagttccagcacttctgcgtttatcatgtgttgacacccatgcaaatgagctgaccctcatggtcatgagctccatttttgttctcatacctctcattctgattctcactacctatggtgccattgcccgggctgtactgagcatgcaatcaaccactgggcttcagaaagtgtttaggacatgtggagcccatcttatggttgtatctctctttttcattccagtcatgtgcatgtatctccagccaccatcagaaaattctcctgatcagggcaagttcattgccctcttttatactgttgtcacaccgagtcttaatcctctaatctacactctcaggaacaaagaagttaaaaaggccataaagaggttgttcaagagaaagtgctgcaggagaaggtga

SEQ ID NO: 2 - protein, 314 aa, synthetic construct
  source 1..314: note = OR2J2 amino acid sequence with an optimized C-terminus
MMIKKNASSEDFFILLGFSNWPQLEVVLFVVILIFYLMTLTGNLFIIILSYVDSHLHTPMYFFLSNLSFLDLCYTTSSIPQLLVNLRGPEKTISYAGCMVQLYFVLALGIAECVLLVVMSYDRYVAVCRPLHYTVLMHPRFCHLLVAASWVIGFTISALHSSFTFWVPLCGHRLVDHFFCEVPALLRLSCVDTHANELTLMVMSSIFVLIPLILILTTYGAIARAVLSMQSTTGLQKVFRTCGAHLMVVSLFFIPVMCMYLQPPSENSPDQGKFIALFYTVVTPSLNPLIYTLRNKEVKKAIKRLFKRKCCRRR

SEQ ID NO: 3 - DNA, 588 bp, synthetic construct
  source 1..588: mol_type = other DNA; note = CMV Promoter
gttgacattgattattgactagttattaatagtaatcaattacggggtcattagttcatagcccatatatggagttccgcgttacataacttacggtaaatggcccgcctggctgaccgcccaacgacccccgcccattgacgtcaataatgacgtatgttcccatagtaacgccaatagggactttccattgacgtcaatgggtggagtatttacggtaaactgcccacttggcagtacatcaagtgtatcatatgccaagtacgccccctattgacgtcaatgacggtaaatggcccgcctggcattatgcccagtacatgaccttatgggactttcctacttggcagtacatctacgtattagtcatcgctattaccatggtgatgcggttttggcagtacatcaatgggcgtggatagcggtttgactcacggggatttccaagtctccaccccattgacgtcaatgggagtttgttttggcaccaaaatcaacgggactttccaaaatgtcgtaacaactccgccccattgacgcaaatgggcggtaggcgtgtacggtgggaggtctatataagcagagctc

SEQ ID NO: 4 - DNA, 225 bp, synthetic construct
  source 1..225: mol_type = other DNA; note = bgh terminator
ctgtgccttctagttgccagccatctgttgtttgcccctcccccgtgccttccttgaccctggaaggtgccactcccactgtcctttcctaataaaatgaggaaattgcatcgcattgtctgagtaggtgtcattctattctggggggtggggtggggcaggacagcaagggggaggattgggaagacaatagcaggcatgctggggatgcggtgggctctatgg

SEQ ID NO: 5 - DNA, 150 bp, synthetic construct
  source 1..150: mol_type = other DNA; note = mmLucy-FLAG-rho
atgagccaccagatcctgctgctcctggccctgctgaccctaggcctggctgattacaaggacgacgacgataagatcgaattgatgaacgggaccgagggcccaaacttctacgtgcctttctccaacaagacgggcgtggtggaattc

SEQ ID NO: 6 - protein, 48 aa, synthetic construct
  source 1..48: note = mmLucy-FLAG-rho
MSHQILLLLALLTLGLAMDYKDDDDKMNGTEGPNFYVPFSNKTGVVEF

SEQ ID NO: 7 - DNA, 684 bp, synthetic construct
  source 1..684: mol_type = other DNA; note = RTP1S(V227I)
atgtgtaaaagcgtgaccacagatgagtggaagaaagtcttctatgagaagatggaggaggcaaagccggctgacagctgggacctcatcatagaccccaacctcaagcacaatgtgctgagccctggttggaagcagtacctggaattgcatgcttcaggcaggttccactgctcctggtgctggcacacctggcagtcgccctacgtggtcatcctcttccacatgttcctggaccgcgcccagcgggcgggctcggtgcgcatgcgcgtcttcaagcagctgtgctatgagtgcggcacggcgcggctggacgagtccagcatgctggaggagaacatcgagggcctggtggacaacctcatcaccagcctgcgcgagcagtgctacggcgagcgtggcggccagtaccgcatccacgtggccagccgccaggacaaccggcggcaccgcggagagttctgcgaggcctgccaggagggcatcgtgcactggaagcccagcgagaagctgctggaggaggaggcgaccacctacaccttctcccgggcgcccagccccaccaagtcgcaggaccagacgggctcaggctggaacttctgctctatcccctggtgcttgttttgggccacggtcctgctgctgatcatctacctgcagttctctttccgtagctccatctaa

SEQ ID NO: 8 - protein, 227 aa, synthetic construct
  source 1..227: note = RTP1S(V227I)
MCKSVTTDEWKKVFYEKMEEAKPADSWDLIIDPNLKHNVLSPGWKQYLELHASGRFHCSWCWHTWQSPYVVILFHMFLDRAQRAGSVRMRVFKQLCYECGTARLDESSMLEENIEGLVDNLITSLREQCYGERGGQYRIHVASRQDNRRHRGEFCEACQEGIVHWKPSEKLLEEEATTYTFSRAPSPTKSQDQTGSGWNFCSIPWCLFWATVLLLIIYLQFSFRSSI

SEQ ID NO: 9 - DNA, 678 bp, synthetic construct
  source 1..678: mol_type = other DNA; note = RTP2(L220R)
atgtgtaccagcttgaccacttgtgagtggaagaaagtcttctatgagaagatggaggtggcaaagccagcggacagctgggagctcatcatagaccccaacctcaagcccagtgagctggcccctggctggaagcagtacctggagcagcacgcctcaggcaggttccactgctcctggtgctggcacacctggcagtctgcccatgtggtcatcctcttccacatgttcctggaccgcgcccagcgggcgggctcggtgcgcatgcgcgtcttcaagcagctgtgctatgagtgcggcacggcgcggctggacgagtccagcatgctggaggagaacatcgagggcctggtggacaacctcatcaccagcctgcgcgagcagtgctacgaggaggatggtggccagtaccgcatccacgtggccagccgcccggacagcgggccgcatcgtgcagagttctgtgaggcctgccaggagggcatcgttcactggaagcccagcgagaagctgctggaggaggaggtgaccacctacacctctgaagcctccaagccgagggcccaggcgggatccggctacaacttcttgtctcttcgctggtgcctcttctgggcctctctctgcctgctcgttgtttacctgcagttctccttccgcagtcctgccttcttttag

SEQ ID NO: 10 - protein, 225 aa, synthetic construct
  source 1..225: note = RTP2(L220R)
MCTSLTTCEWKKVFYEKMEVAKPADSWELIIDPNLKPSELAPGWKQYLEQHASGRFHCSWCWHTWQSAHVVILFHMFLDRAQRAGSVRMRVFKQLCYECGTARLDESSMLEENIEGLVDNLITSLREQCYEEDGGQYRIHVASRPDSGPHRAEFCEACQEGIVHWKPSEKLLEEEVTTYTSEASKPRAQAGSGYNFLSLRWCLFWASLCLLVVYLQFSFRSPAFF